European Patent Application EP 4 115 893 A1, published January 11, 2023. Title: Anti-tumor composition. Applicant: Shanghai Sine Pharmaceutical Laboratories Co., Ltd. The sequence listing filed with the application follows.

SEQUENCE LISTING (1 sequence)

SEQ ID NO: 1 - DNA, 1414 bp, Akkermansia muciniphila
cccagtgggcggcgtcaagacatgcaagtcgacgagagaattgctagcttgctaataattcctctagtggcgcacgggtgagtaacacgtgagtaacctgcccccgagagcgggatagccctgggaaactgggattaataccgcatagtatcgaaagattaaagcagcaatgcgcttggggatgggctcgcggcctattagttagttggtgaggtaacggctcaccaaggcgatgacgggtagccggtctgagaggatgtccggccacactggaactgagacacggtccagacacctacgggtggcagcagtcgagaatcattcacaatgggggaaaccctgatggtgcgacgccgcgtgggggaatgaaggtcttcggattgtaaacccctgtcatgtgggagcaaattaaaaagatagtaccacaagaggaagagacggctaactctgtgccagcagccgcggtaatacagaggtctcaagcgttgttcggaatcactgggcgtaaagcgtgcgtaggctgtttcgtaagtcgtgtgtgaaaggcgcgggctcaacccgcggacggcacatgatactgcgagactagagtaatggagggggaaccggaattctcggtgtagcagtgaaatgcgtagatatcgagaggaacactcgtggcgaaggcgggttcctggacattaactgacgctgaggcacgaaggccaggggagcgaaagggattagatacccctgtagtcctggcagtaaacggtgcacgcttggtgtgcggggaatcgaccccctgcgtgccggagctaacgcgttaagcgtgccgcctggggagtacggtcgcaagattaaaactcaaagaaattgacggggacccgcacaagcggtggagtatgtggcttaattcgatgcaacgcgaagaaccttacctgggcttgacatgtaatgaacaacatgtgaaagcatgcgactcttcggaggcgttacacaggtgctgcatggccgtcgtcagctcgtgtcgtgagatgtttggttaagtccagcaacgagcgcaacccctgttgccagttaccagcacgtgaaggtggggactctggcgagactgcccagatcaactgggaggaaggtggggacgacgtcaggtcagtatggcccttatgcccagggctgcacacgtactacaatgcccagtacagagggggccgaagccgcgaggcggaggaaatcctaaaaactgggcccagttcggactgtaggctgcaacccgcctacacgaagccggaatcgctagtaatggcgcatcagctacggcgccgtgaatacgttcccgggtcttgtacacaccgcccgtcacatcatggaagccggtcgcacccgaagtatctgaagccaaccgcaaggaggcaggtctaagtagactggt